European Patent Specification EP 3 706 777 B1, published May 22, 2024. Title: ACTIVIN RECEPTOR TYPE IIA VARIANTS AND METHODS OF USE THEREOF. Applicant: Keros Therapeutics, Inc. The sequence listing filed with the application follows.

SEQUENCE LISTING (155 sequences)

SEQ ID NO: 1 - protein, 109 aa, Artificial Sequence
  Synthetic Construct
  MISC_FEATURE (14)..(14): Xaa is Phe or Tyr
  MISC_FEATURE (15)..(15): Xaa is Phe or Tyr
  MISC_FEATURE (20)..(20): Xaa is Glu or Ala
  MISC_FEATURE (21)..(21): Xaa is Lys or Leu
  MISC_FEATURE (22)..(22): Xaa is Asp or Glu
  MISC_FEATURE (23)..(23): Xaa is Arg or Ala
  MISC_FEATURE (31)..(31): Xaa is Pro or Arg
  MISC_FEATURE (33)..(33): Xaa is Tyr or Glu
  MISC_FEATURE (35)..(35): Xaa is Asp or Glu
  MISC_FEATURE (36)..(36): Xaa is Lys or Gln
  MISC_FEATURE (37)..(37): Xaa is Asp or Ala
  MISC_FEATURE (38)..(38): Xaa is Lys or Ala
  MISC_FEATURE (39)..(39): Xaa is Arg or Ala
  MISC_FEATURE (40)..(40): Xaa is Arg or Leu
  MISC_FEATURE (43)..(43): Xaa is Phe or Tyr
  MISC_FEATURE (47)..(47): Xaa is Lys, Arg, or Ala
  MISC_FEATURE (57)..(57): Xaa is Lys, Ala, Tyr, Phe, or Ile
  MISC_FEATURE (58)..(58): Xaa is Gln or Lys
  MISC_FEATURE (61)..(61): Xaa is Trp or Ala
  MISC_FEATURE (62)..(62): Xaa is Leu or Ala
  MISC_FEATURE (63)..(63): Xaa is Asp, Lys, Arg, Ala, Phe, Gly, Met, Asn, or Ile
  MISC_FEATURE (65)..(65): Xaa is Ile, Phe, or Ala
  MISC_FEATURE (76)..(76): Xaa is Lys or Thr
  MISC_FEATURE (77)..(77): Xaa is Lys or Glu
  MISC_FEATURE (78)..(78): Xaa is Asp or Glu
  MISC_FEATURE (79)..(79): Xaa is Ser or Asn
  MISC_FEATURE (81)..(81): Xaa is Glu or Gln
GAILGRSETQECLXXNANWXXXXTNQTGVEXCXGXXXXXXHCXATWXNISGSIEIVXXGCXXXDXNCYDRTDCVEXXXXPXVYFCCCEGNMCNEKFSYFPEMEVTQPTS

SEQ ID NO: 2 - protein, 109 aa, Artificial Sequence
  Synthetic Construct
  MISC_FEATURE (15)..(15): Xaa is Phe or Tyr
  MISC_FEATURE (20)..(20): Xaa is Glu or Ala
  MISC_FEATURE (21)..(21): Xaa is Lys or Leu
  MISC_FEATURE (22)..(22): Xaa is Asp or Glu
  MISC_FEATURE (23)..(23): Xaa is Arg or Ala
  MISC_FEATURE (31)..(31): Xaa is Pro or Arg
  MISC_FEATURE (33)..(33): Xaa is Tyr or Glu
  MISC_FEATURE (35)..(35): Xaa is Asp or Glu
  MISC_FEATURE (37)..(37): Xaa is Asp or Ala
  MISC_FEATURE (38)..(38): Xaa is Lys or Ala
  MISC_FEATURE (39)..(39): Xaa is Arg or Ala
  MISC_FEATURE (40)..(40): Xaa is Arg or Leu
  MISC_FEATURE (43)..(43): Xaa is Phe or Tyr
  MISC_FEATURE (47)..(47): Xaa is Lys, Arg, or Ala
  MISC_FEATURE (57)..(57): Xaa is Lys, Ala, Tyr, Phe, or Ile
  MISC_FEATURE (58)..(58): Xaa is Gln or Lys
  MISC_FEATURE (61)..(61): Xaa is Trp or Ala
  MISC_FEATURE (62)..(62): Xaa is Leu or Ala
  MISC_FEATURE (63)..(63): Xaa is Asp, Lys, Arg, Ala, Phe, Gly, Met, Asn, or Ile
  MISC_FEATURE (65)..(65): Xaa is Ile, Phe, or Ala
  MISC_FEATURE (76)..(76): Xaa is Lys or Thr
  MISC_FEATURE (77)..(77): Xaa is Lys or Glu
  MISC_FEATURE (78)..(78): Xaa is Asp or Glu
  MISC_FEATURE (79)..(79): Xaa is Ser or Asn
  MISC_FEATURE (81)..(81): Xaa is Glu or Gln
GAILGRSETQECLFXNANWXXXXTNQTGVEXCXGXKXXXXHCXATWXNISGSIEIVXXGCXXXDXNCYDRTDCVEXXXXPXVYFCCCEGNMCNEKFSYFPEMEVTQPTS

SEQ ID NO: 3 - protein, 109 aa, Artificial Sequence
  Synthetic Construct
  MISC_FEATURE (15)..(15): Xaa is Phe or Tyr
  MISC_FEATURE (21)..(21): Xaa is Lys or Leu
  MISC_FEATURE (22)..(22): Xaa is Asp or Glu
  MISC_FEATURE (31)..(31): Xaa is Pro or Arg
  MISC_FEATURE (33)..(33): Xaa is Tyr or Glu
  MISC_FEATURE (35)..(35): Xaa is Asp or Glu
  MISC_FEATURE (40)..(40): Xaa is Arg or Leu
  MISC_FEATURE (43)..(43): Xaa is Phe or Tyr
  MISC_FEATURE (47)..(47): Xaa is Lys, Arg, or Ala
  MISC_FEATURE (58)..(58): Xaa is Gln or Lys
  MISC_FEATURE (65)..(65): Xaa is Ile, Phe, or Ala
  MISC_FEATURE (76)..(76): Xaa is Lys or Thr
  MISC_FEATURE (77)..(77): Xaa is Lys or Glu
  MISC_FEATURE (78)..(78): Xaa is Asp or Glu
  MISC_FEATURE (79)..(79): Xaa is Ser or Asn
  MISC_FEATURE (81)..(81): Xaa is Glu or Gln
GAILGRSETQECLFXNANWEXXRTNQTGVEXCXGXKDKRXHCXATWXNISGSIEIVKXGCWLDDXNCYDRTDCVEXXXXPXVYFCCCEGNMCNEKFSYFPEMEVTQPTS

SEQ ID NO: 4 - protein, 109 aa, Artificial Sequence
  Synthetic Construct
  MISC_FEATURE (15)..(15): Xaa is Phe or Tyr
  MISC_FEATURE (21)..(21): Xaa is Lys or Leu
  MISC_FEATURE (31)..(31): Xaa is Pro or Arg
  MISC_FEATURE (33)..(33): Xaa is Tyr or Glu
  MISC_FEATURE (35)..(35): Xaa is Asp or Glu
  MISC_FEATURE (40)..(40): Xaa is Arg or Leu
  MISC_FEATURE (43)..(43): Xaa is Phe or Tyr
  MISC_FEATURE (47)..(47): Xaa is Lys, Arg, or Ala
  MISC_FEATURE (58)..(58): Xaa is Gln or Lys
  MISC_FEATURE (65)..(65): Xaa is Ile, Phe, or Ala
  MISC_FEATURE (76)..(76): Xaa is Lys or Thr
  MISC_FEATURE (78)..(78): Xaa is Asp or Glu
  MISC_FEATURE (79)..(79): Xaa is Ser or Asn
  MISC_FEATURE (81)..(81): Xaa is Glu or Gln
GAILGRSETQECLFXNANWEXDRTNQTGVEXCXGXKDKRXHCXATWXNISGSIEIVKXGCWLDDXNCYDRTDCVEXKXXPXVYFCCCEGNMCNEKFSYFPEMEVTQPTS

SEQ ID NO: 5 - protein, 109 aa, Artificial Sequence
  Synthetic Construct
  MISC_FEATURE (15)..(15): Xaa is Phe or Tyr
  MISC_FEATURE (21)..(21): Xaa is Lys or Leu
  MISC_FEATURE (33)..(33): Xaa is Tyr or Glu
  MISC_FEATURE (35)..(35): Xaa is Asp or Glu
  MISC_FEATURE (40)..(40): Xaa is Arg or Leu
  MISC_FEATURE (58)..(58): Xaa is Gln or Lys
  MISC_FEATURE (76)..(76): Xaa is Lys or Thr
  MISC_FEATURE (78)..(78): Xaa is Asp or Glu
  MISC_FEATURE (79)..(79): Xaa is Ser or Asn
  MISC_FEATURE (81)..(81): Xaa is Glu or Gln
GAILGRSETQECLFXNANWEXDRTNQTGVEPCXGXKDKRXHCFATWKNISGSIEIVKXGCWLDDINCYDRTDCVEXKXXPXVYFCCCEGNMCNEKFSYFPEMEVTQPTS

SEQ ID NO: 6 - protein, 109 aa, Artificial Sequence
  Synthetic Construct
GAILGRSETQECLFYNANWELDRTNQTGVEPCEGEKDKRLHCFATWKNISGSIEIVKKGCWLDDINCYDRTDCVETKENPQVYFCCCEGNMCNEKFSYFPEMEVTQPTS

SEQ ID NO: 7 - protein, 109 aa, Artificial Sequence
  Synthetic Construct
GAILGRSETQECLFYNANWELERTNQTGVEPCEGEKDKRLHCFATWKNISGSIEIVKKGCWLDDINCYDRTDCVETKENPQVYFCCCEGNMCNEKFSYFPEMEVTQPTS

SEQ ID NO: 8 - protein, 109 aa, Artificial Sequence
  Synthetic Construct
GAILGRSETQECLFYNANWELDRTNQTGVERCEGEKDKRLHCFATWKNISGSIEIVKKGCWLDDINCYDRTDCVETKENPQVYFCCCEGNMCNEKFSYFPEMEVTQPTS

SEQ ID NO: 9 - protein, 109 aa, Artificial Sequence
  Synthetic Construct
GAILGRSETQECLFYNANWELDRTNQTGVEPCEGEKDKRLHCYATWKNISGSIEIVKKGCWLDDINCYDRTDCVETKENPQVYFCCCEGNMCNEKFSYFPEMEVTQPTS

SEQ ID NO: 10 - protein, 109 aa, Artificial Sequence
  Synthetic Construct
GAILGRSETQECLFYNANWELDRTNQTGVEPCEGEKDKRLHCFATWRNISGSIEIVKKGCWLDDINCYDRTDCVETKENPQVYFCCCEGNMCNEKFSYFPEMEVTQPTS

SEQ ID NO: 11 - protein, 109 aa, Artificial Sequence
  Synthetic Construct
GAILGRSETQECLFYNANWELDRTNQTGVEPCEGEKDKRLHCFATWKNISGSIEIVKKGCWLDDFNCYDRTDCVETKENPQVYFCCCEGNMCNEKFSYFPEMEVTQPTS

SEQ ID NO: 12 - protein, 109 aa, Artificial Sequence
  Synthetic Construct
GAILGRSETQECLFYNANWELDRTNQTGVEPCEGEKDKRLHCFATWKNISGSIEIVKKGCWLDDINCYDRTDCVETEENPQVYFCCCEGNMCNEKFSYFPEMEVTQPTS

SEQ ID NO: 13 - protein, 109 aa, Artificial Sequence
  Synthetic Construct
GAILGRSETQECLFYNANWELERTNQTGVERCEGEKDKRLHCFATWKNISGSIEIVKKGCWLDDINCYDRTDCVETKENPQVYFCCCEGNMCNEKFSYFPEMEVTQPTS

SEQ ID NO: 14 - protein, 109 aa, Artificial Sequence
  Synthetic Construct
GAILGRSETQECLFYNANWELERTNQTGVEPCEGEKDKRLHCYATWKNISGSIEIVKKGCWLDDINCYDRTDCVETKENPQVYFCCCEGNMCNEKFSYFPEMEVTQPTS

SEQ ID NO: 15 - protein, 109 aa, Artificial Sequence
  Synthetic Construct
GAILGRSETQECLFYNANWELERTNQTGVEPCEGEKDKRLHCFATWRNISGSIEIVKKGCWLDDINCYDRTDCVETKENPQVYFCCCEGNMCNEKFSYFPEMEVTQPTS

SEQ ID NO: 16 - protein, 109 aa, Artificial Sequence
  Synthetic Construct
GAILGRSETQECLFYNANWELERTNQTGVEPCEGEKDKRLHCFATWKNISGSIEIVKKGCWLDDFNCYDRTDCVETKENPQVYFCCCEGNMCNEKFSYFPEMEVTQPTS

SEQ ID NO: 17 - protein, 109 aa, Artificial Sequence
  Synthetic Construct
GAILGRSETQECLFYNANWELERTNQTGVEPCEGEKDKRLHCFATWKNISGSIEIVKKGCWLDDINCYDRTDCVETEENPQVYFCCCEGNMCNEKFSYFPEMEVTQPTS

SEQ ID NO: 18 - protein, 109 aa, Artificial Sequence
  Synthetic Construct
GAILGRSETQECLFYNANWELDRTNQTGVERCEGEKDKRLHCYATWKNISGSIEIVKKGCWLDDINCYDRTDCVETKENPQVYFCCCEGNMCNEKFSYFPEMEVTQPTS

SEQ ID NO: 19 - protein, 109 aa, Artificial Sequence
  Synthetic Construct
GAILGRSETQECLFYNANWELDRTNQTGVERCEGEKDKRLHCFATWRNISGSIEIVKKGCWLDDINCYDRTDCVETKENPQVYFCCCEGNMCNEKFSYFPEMEVTQPTS

SEQ ID NO: 20 - protein, 109 aa, Artificial Sequence
  Synthetic Construct
GAILGRSETQECLFYNANWELDRTNQTGVERCEGEKDKRLHCFATWKNISGSIEIVKKGCWLDDFNCYDRTDCVETKENPQVYFCCCEGNMCNEKFSYFPEMEVTQPTS

SEQ ID NO: 21 - protein, 109 aa, Artificial Sequence
  Synthetic Construct
GAILGRSETQECLFYNANWELDRTNQTGVERCEGEKDKRLHCFATWKNISGSIEIVKKGCWLDDINCYDRTDCVETEENPQVYFCCCEGNMCNEKFSYFPEMEVTQPTS

SEQ ID NO: 22 - protein, 109 aa, Artificial Sequence
  Synthetic Construct
GAILGRSETQECLFYNANWELDRTNQTGVEPCEGEKDKRLHCYATWRNISGSIEIVKKGCWLDDINCYDRTDCVETKENPQVYFCCCEGNMCNEKFSYFPEMEVTQPTS

SEQ ID NO: 23 - protein, 109 aa, Artificial Sequence
  Synthetic Construct
GAILGRSETQECLFYNANWELDRTNQTGVEPCEGEKDKRLHCYATWKNISGSIEIVKKGCWLDDFNCYDRTDCVETKENPQVYFCCCEGNMCNEKFSYFPEMEVTQPTS

SEQ ID NO: 24 - protein, 109 aa, Artificial Sequence
  Synthetic Construct
GAILGRSETQECLFYNANWELDRTNQTGVEPCEGEKDKRLHCYATWKNISGSIEIVKKGCWLDDINCYDRTDCVETEENPQVYFCCCEGNMCNEKFSYFPEMEVTQPTS

SEQ ID NO: 25 - protein, 109 aa, Artificial Sequence
  Synthetic Construct
GAILGRSETQECLFYNANWELDRTNQTGVEPCEGEKDKRLHCFATWRNISGSIEIVKKGCWLDDFNCYDRTDCVETKENPQVYFCCCEGNMCNEKFSYFPEMEVTQPTS

SEQ ID NO: 26 - protein, 109 aa, Artificial Sequence
  Synthetic Construct
GAILGRSETQECLFYNANWELDRTNQTGVEPCEGEKDKRLHCFATWRNISGSIEIVKKGCWLDDINCYDRTDCVETEENPQVYFCCCEGNMCNEKFSYFPEMEVTQPTS

SEQ ID NO: 27 - protein, 109 aa, Artificial Sequence
  Synthetic Construct
GAILGRSETQECLFYNANWELDRTNQTGVEPCEGEKDKRLHCFATWKNISGSIEIVKKGCWLDDFNCYDRTDCVETEENPQVYFCCCEGNMCNEKFSYFPEMEVTQPTS

SEQ ID NO: 28 - protein, 109 aa, Artificial Sequence
  Synthetic Construct
GAILGRSETQECLFYNANWELERTNQTGVERCEGEKDKRLHCYATWKNISGSIEIVKKGCWLDDINCYDRTDCVETKENPQVYFCCCEGNMCNEKFSYFPEMEVTQPTS

SEQ ID NO: 29 - protein, 109 aa, Artificial Sequence
  Synthetic Construct
GAILGRSETQECLFYNANWELERTNQTGVERCEGEKDKRLHCFATWRNISGSIEIVKKGCWLDDINCYDRTDCVETKENPQVYFCCCEGNMCNEKFSYFPEMEVTQPTS

SEQ ID NO: 30 - protein, 109 aa, Artificial Sequence
  Synthetic Construct
GAILGRSETQECLFYNANWELERTNQTGVERCEGEKDKRLHCFATWKNISGSIEIVKKGCWLDDFNCYDRTDCVETKENPQVYFCCCEGNMCNEKFSYFPEMEVTQPTS

SEQ ID NO: 31 - protein, 109 aa, Artificial Sequence
  Synthetic Construct
GAILGRSETQECLFYNANWELERTNQTGVERCEGEKDKRLHCFATWKNISGSIEIVKKGCWLDDINCYDRTDCVETEENPQVYFCCCEGNMCNEKFSYFPEMEVTQPTS

SEQ ID NO: 32 - protein, 109 aa, Artificial Sequence
  Synthetic Construct
GAILGRSETQECLFYNANWELERTNQTGVEPCEGEKDKRLHCYATWRNISGSIEIVKKGCWLDDINCYDRTDCVETKENPQVYFCCCEGNMCNEKFSYFPEMEVTQPTS

SEQ ID NO: 33 - protein, 109 aa, Artificial Sequence
  Synthetic Construct
GAILGRSETQECLFYNANWELERTNQTGVEPCEGEKDKRLHCYATWKNISGSIEIVKKGCWLDDFNCYDRTDCVETKENPQVYFCCCEGNMCNEKFSYFPEMEVTQPTS

SEQ ID NO: 34 - protein, 109 aa, Artificial Sequence
  Synthetic Construct
GAILGRSETQECLFYNANWELERTNQTGVEPCEGEKDKRLHCYATWKNISGSIEIVKKGCWLDDINCYDRTDCVETEENPQVYFCCCEGNMCNEKFSYFPEMEVTQPTS

SEQ ID NO: 35 - protein, 109 aa, Artificial Sequence
  Synthetic Construct
GAILGRSETQECLFYNANWELERTNQTGVEPCEGEKDKRLHCFATWRNISGSIEIVKKGCWLDDFNCYDRTDCVETKENPQVYFCCCEGNMCNEKFSYFPEMEVTQPTS

SEQ ID NO: 36 - protein, 109 aa, Artificial Sequence
  Synthetic Construct
GAILGRSETQECLFYNANWELERTNQTGVEPCEGEKDKRLHCFATWRNISGSIEIVKKGCWLDDINCYDRTDCVETEENPQVYFCCCEGNMCNEKFSYFPEMEVTQPTS

SEQ ID NO: 37 - protein, 109 aa, Artificial Sequence
  Synthetic Construct
GAILGRSETQECLFYNANWELERTNQTGVEPCEGEKDKRLHCFATWKNISGSIEIVKKGCWLDDFNCYDRTDCVETEENPQVYFCCCEGNMCNEKFSYFPEMEVTQPTS

SEQ ID NO: 38 - protein, 109 aa, Artificial Sequence
  Synthetic Construct
GAILGRSETQECLFYNANWELDRTNQTGVERCEGEKDKRLHCYATWRNISGSIEIVKKGCWLDDINCYDRTDCVETKENPQVYFCCCEGNMCNEKFSYFPEMEVTQPTS

SEQ ID NO: 39 - protein, 109 aa, Artificial Sequence
  Synthetic Construct
GAILGRSETQECLFYNANWELDRTNQTGVERCEGEKDKRLHCYATWKNISGSIEIVKKGCWLDDFNCYDRTDCVETKENPQVYFCCCEGNMCNEKFSYFPEMEVTQPTS

SEQ ID NO: 40 - protein, 109 aa, Artificial Sequence
  Synthetic Construct
GAILGRSETQECLFYNANWELDRTNQTGVERCEGEKDKRLHCYATWKNISGSIEIVKKGCWLDDINCYDRTDCVETEENPQVYFCCCEGNMCNEKFSYFPEMEVTQPTS

SEQ ID NO: 41 - protein, 109 aa, Artificial Sequence
  Synthetic Construct
GAILGRSETQECLFYNANWELDRTNQTGVERCEGEKDKRLHCFATWRNISGSIEIVKKGCWLDDFNCYDRTDCVETKENPQVYFCCCEGNMCNEKFSYFPEMEVTQPTS

SEQ ID NO: 42 - protein, 109 aa, Artificial Sequence
  Synthetic Construct
GAILGRSETQECLFYNANWELDRTNQTGVERCEGEKDKRLHCFATWRNISGSIEIVKKGCWLDDINCYDRTDCVETEENPQVYFCCCEGNMCNEKFSYFPEMEVTQPTS

SEQ ID NO: 43 - protein, 109 aa, Artificial Sequence
  Synthetic Construct
GAILGRSETQECLFYNANWELDRTNQTGVERCEGEKDKRLHCFATWKNISGSIEIVKKGCWLDDFNCYDRTDCVETEENPQVYFCCCEGNMCNEKFSYFPEMEVTQPTS

SEQ ID NO: 44 - protein, 109 aa, Artificial Sequence
  Synthetic Construct
GAILGRSETQECLFYNANWELDRTNQTGVEPCEGEKDKRLHCYATWRNISGSIEIVKKGCWLDDFNCYDRTDCVETKENPQVYFCCCEGNMCNEKFSYFPEMEVTQPTS

SEQ ID NO: 45 - protein, 109 aa, Artificial Sequence
  Synthetic Construct
GAILGRSETQECLFYNANWELDRTNQTGVEPCEGEKDKRLHCYATWRNISGSIEIVKKGCWLDDINCYDRTDCVETEENPQVYFCCCEGNMCNEKFSYFPEMEVTQPTS

SEQ ID NO: 46 - protein, 109 aa, Artificial Sequence
  Synthetic Construct
GAILGRSETQECLFYNANWELDRTNQTGVEPCEGEKDKRLHCYATWKNISGSIEIVKKGCWLDDFNCYDRTDCVETEENPQVYFCCCEGNMCNEKFSYFPEMEVTQPTS

SEQ ID NO: 47 - protein, 109 aa, Artificial Sequence
  Synthetic Construct
GAILGRSETQECLFYNANWELDRTNQTGVEPCEGEKDKRLHCFATWRNISGSIEIVKKGCWLDDFNCYDRTDCVETEENPQVYFCCCEGNMCNEKFSYFPEMEVTQPTS

SEQ ID NO: 48 - protein, 109 aa, Artificial Sequence
  Synthetic Construct
GAILGRSETQECLFYNANWELERTNQTGVERCEGEKDKRLHCYATWRNISGSIEIVKKGCWLDDINCYDRTDCVETKENPQVYFCCCEGNMCNEKFSYFPEMEVTQPTS

SEQ ID NO: 49 - protein, 109 aa, Artificial Sequence
  Synthetic Construct
GAILGRSETQECLFYNANWELERTNQTGVERCEGEKDKRLHCYATWKNISGSIEIVKKGCWLDDFNCYDRTDCVETKENPQVYFCCCEGNMCNEKFSYFPEMEVTQPTS

SEQ ID NO: 50 - protein, 109 aa, Artificial Sequence
  Synthetic Construct
GAILGRSETQECLFYNANWELERTNQTGVERCEGEKDKRLHCYATWKNISGSIEIVKKGCWLDDINCYDRTDCVETEENPQVYFCCCEGNMCNEKFSYFPEMEVTQPTS

SEQ ID NO: 51 - protein, 109 aa, Artificial Sequence
  Synthetic Construct
GAILGRSETQECLFYNANWELERTNQTGVERCEGEKDKRLHCFATWRNISGSIEIVKKGCWLDDFNCYDRTDCVETKENPQVYFCCCEGNMCNEKFSYFPEMEVTQPTS

SEQ ID NO: 52 - protein, 109 aa, Artificial Sequence
  Synthetic Construct
GAILGRSETQECLFYNANWELERTNQTGVERCEGEKDKRLHCFATWRNISGSIEIVKKGCWLDDINCYDRTDCVETEENPQVYFCCCEGNMCNEKFSYFPEMEVTQPTS

SEQ ID NO: 53 - protein, 109 aa, Artificial Sequence
  Synthetic Construct
GAILGRSETQECLFYNANWELERTNQTGVERCEGEKDKRLHCFATWKNISGSIEIVKKGCWLDDFNCYDRTDCVETEENPQVYFCCCEGNMCNEKFSYFPEMEVTQPTS

SEQ ID NO: 54 - protein, 109 aa, Artificial Sequence
  Synthetic Construct
GAILGRSETQECLFYNANWELERTNQTGVEPCEGEKDKRLHCYATWRNISGSIEIVKKGCWLDDFNCYDRTDCVETKENPQVYFCCCEGNMCNEKFSYFPEMEVTQPTS

SEQ ID NO: 55 - protein, 109 aa, Artificial Sequence
  Synthetic Construct
GAILGRSETQECLFYNANWELERTNQTGVEPCEGEKDKRLHCYATWRNISGSIEIVKKGCWLDDINCYDRTDCVETEENPQVYFCCCEGNMCNEKFSYFPEMEVTQPTS

SEQ ID NO: 56 - protein, 109 aa, Artificial Sequence
  Synthetic Construct
GAILGRSETQECLFYNANWELERTNQTGVEPCEGEKDKRLHCYATWKNISGSIEIVKKGCWLDDFNCYDRTDCVETEENPQVYFCCCEGNMCNEKFSYFPEMEVTQPTS

SEQ ID NO: 57 - protein, 109 aa, Artificial Sequence
  Synthetic Construct
GAILGRSETQECLFYNANWELERTNQTGVEPCEGEKDKRLHCFATWRNISGSIEIVKKGCWLDDFNCYDRTDCVETEENPQVYFCCCEGNMCNEKFSYFPEMEVTQPTS

SEQ ID NO: 58 - protein, 109 aa, Artificial Sequence
  Synthetic Construct
GAILGRSETQECLFYNANWELDRTNQTGVERCEGEKDKRLHCYATWRNISGSIEIVKKGCWLDDFNCYDRTDCVETKENPQVYFCCCEGNMCNEKFSYFPEMEVTQPTS

SEQ ID NO: 59 - protein, 109 aa, Artificial Sequence
  Synthetic Construct
GAILGRSETQECLFYNANWELDRTNQTGVERCEGEKDKRLHCYATWRNISGSIEIVKKGCWLDDINCYDRTDCVETEENPQVYFCCCEGNMCNEKFSYFPEMEVTQPTS

SEQ ID NO: 60 - protein, 109 aa, Artificial Sequence
  Synthetic Construct
GAILGRSETQECLFYNANWELDRTNQTGVERCEGEKDKRLHCYATWKNISGSIEIVKKGCWLDDFNCYDRTDCVETEENPQVYFCCCEGNMCNEKFSYFPEMEVTQPTS

SEQ ID NO: 61 - protein, 109 aa, Artificial Sequence
  Synthetic Construct
GAILGRSETQECLFYNANWELDRTNQTGVERCEGEKDKRLHCFATWRNISGSIEIVKKGCWLDDFNCYDRTDCVETEENPQVYFCCCEGNMCNEKFSYFPEMEVTQPTS

SEQ ID NO: 62 - protein, 109 aa, Artificial Sequence
  Synthetic Construct
GAILGRSETQECLFYNANWELDRTNQTGVEPCEGEKDKRLHCYATWRNISGSIEIVKKGCWLDDFNCYDRTDCVETEENPQVYFCCCEGNMCNEKFSYFPEMEVTQPTS

SEQ ID NO: 63 - protein, 109 aa, Artificial Sequence
  Synthetic Construct
GAILGRSETQECLFYNANWELERTNQTGVERCEGEKDKRLHCYATWRNISGSIEIVKKGCWLDDFNCYDRTDCVETKENPQVYFCCCEGNMCNEKFSYFPEMEVTQPTS

SEQ ID NO: 64 - protein, 109 aa, Artificial Sequence
  Synthetic Construct
GAILGRSETQECLFYNANWELERTNQTGVERCEGEKDKRLHCYATWRNISGSIEIVKKGCWLDDINCYDRTDCVETEENPQVYFCCCEGNMCNEKFSYFPEMEVTQPTS

SEQ ID NO: 65 - protein, 109 aa, Artificial Sequence
  Synthetic Construct
GAILGRSETQECLFYNANWELERTNQTGVERCEGEKDKRLHCYATWKNISGSIEIVKKGCWLDDFNCYDRTDCVETEENPQVYFCCCEGNMCNEKFSYFPEMEVTQPTS

SEQ ID NO: 66 - protein, 109 aa, Artificial Sequence
  Synthetic Construct
GAILGRSETQECLFYNANWELERTNQTGVERCEGEKDKRLHCFATWRNISGSIEIVKKGCWLDDFNCYDRTDCVETEENPQVYFCCCEGNMCNEKFSYFPEMEVTQPTS

SEQ ID NO: 67 - protein, 109 aa, Artificial Sequence
  Synthetic Construct
GAILGRSETQECLFYNANWELDRTNQTGVERCEGEKDKRLHCYATWRNISGSIEIVKKGCWLDDFNCYDRTDCVETEENPQVYFCCCEGNMCNEKFSYFPEMEVTQPTS

SEQ ID NO: 68 - protein, 109 aa, Artificial Sequence
  Synthetic Construct
GAILGRSETQECLFYNANWELERTNQTGVEPCEGEKDKRLHCYATWRNISGSIEIVKKGCWLDDFNCYDRTDCVETEENPQVYFCCCEGNMCNEKFSYFPEMEVTQPTS

SEQ ID NO: 69 - protein, 109 aa, Artificial Sequence
  Synthetic Construct
GAILGRSETQECLFYNANWELERTNQTGVERCEGEKDKRLHCYATWRNISGSIEIVKKGCWLDDFNCYDRTDCVETEENPQVYFCCCEGNMCNEKFSYFPEMEVTQPTS

SEQ ID NO: 70 - protein, 109 aa, Artificial Sequence
  Synthetic Construct
GAILGRSETQECLYYNANWELERTNQTGVERCEGEQDKRLHCYATWRNISGSIEIVKKGCWLDDFNCYDRTDCVETEENPQVYFCCCEGNMCNEKFSYFPEMEVTQPTS

SEQ ID NO: 71 - protein, 111 aa, Artificial Sequence
  Synthetic Construct
GAILGRSETQECLFYNANWELERTNQTGVERCEGEKDKRLHCYATWRNISGSIEIVKKGCWLDDFNCYDRTDCVETEENPQVYFCCCEGNMCNEKFSYFPEMEVTQPTSNP

SEQ ID NO: 72 - protein, 115 aa, Artificial Sequence
  Synthetic Construct
GAILGRSETQECLFYNANWELERTNQTGVERCEGEKDKRLHCYATWRNISGSIEIVKKGCWLDDFNCYDRTDCVETEENPQVYFCCCEGNMCNEKFSYFPEMEVTQPTSNPVTPK

SEQ ID NO: 73 - protein, 109 aa, Homo sapiens
GAILGRSETQECLFFNANWEKDRTNQTGVEPCYGDKDKRRHCFATWKNISGSIEIVKQGCWLDDINCYDRTDCVEKKDSPEVYFCCCEGNMCNEKFSYFPEMEVTQPTS

SEQ ID NO: 74 - protein, 115 aa, Homo sapiens
GRGEAETRECIYYNANWELERTNQSGLERCEGEQDKRLHCYASWRNSSGTIELVKKGCWLDDFNCYDRQECVATEENPQVYFCCCEGNFCNERFTHLPEAGGPEVTYEPPPTAPT

SEQ ID NO: 75 - protein, 513 aa, Homo sapiens
MGAAAKLAFAVFLISCSSGAILGRSETQECLFFNANWEKDRTNQTGVEPCYGDKDKRRHCFATWKNISGSIEIVKQGCWLDDINCYDRTDCVEKKDSPEVYFCCCEGNMCNEKFSYFPEMEVTQPTSNPVTPKPPYYNILLYSLVPLMLIAGIVICAFWVYRHHKMAYPPVLVPTQDPGPPPPSPLLGLKPLQLLEVKARGRFGCVWKAQLLNEYVAVKIFPIQDKQSWQNEYEVYSLPGMKHENILQFIGAEKRGTSVDVDLWLITAFHEKGSLSDFLKANVVSWNELCHIAETMARGLAYLHEDIPGLKDGHKPAISHRDIKSKNVLLKNNLTACIADFGLALKFEAGKSAGDTHGQVGTRRYMAPEVLEGAINFQRDAFLRIDMYAMGLVLWELASRCTAADGPVDEYMLPFEEEIGQHPSLEDMQEVVVHKKKRPVLRDYWQKHAGMAMLCETIEECWDHDAEARLSAGCVGERITQMQRLTNIITTEDIVTVVTMVTNVDFPPKESSL

SEQ ID NO: 76 - protein, 109 aa, Artificial Sequence
  Synthetic Construct
GAILGRSETQECLFFNANWEKDRTNQTGVEPCYGDKDKRRHCFATWANISGSIEIVKQGCWLDDINCYDRTDCVEKKDSPEVYFCCCEGNMCNEKFSYFPEMEVTQPTS

SEQ ID NO: 77 - protein, 109 aa, Artificial Sequence
  Synthetic Construct
GAILGRSETQECLFFNANWAKDRTNQTGVEPCYGDKDKRRHCFATWKNISGSIEIVKQGCWLDDINCYDRTDCVEKKDSPEVYFCCCEGNMCNEKFSYFPEMEVTQPTS

SEQ ID NO: 78 - protein, 109 aa, Artificial Sequence
  Synthetic Construct
GAILGRSETQECLFFNANWEKDATNQTGVEPCYGDKDKRRHCFATWKNISGSIEIVKQGCWLDDINCYDRTDCVEKKDSPEVYFCCCEGNMCNEKFSYFPEMEVTQPTS

SEQ ID NO: 79 - protein, 109 aa, Artificial Sequence
  Synthetic Construct
GAILGRSETQECLFFNANWEKDRTNQTGVEPCYGDKAKRRHCFATWKNISGSIEIVKQGCWLDDINCYDRTDCVEKKDSPEVYFCCCEGNMCNEKFSYFPEMEVTQPTS

SEQ ID NO: 80 - protein, 109 aa, Artificial Sequence
  Synthetic Construct
GAILGRSETQECLFFNANWEKDRTNQTGVEPCYGDKDARRHCFATWKNISGSIEIVKQGCWLDDINCYDRTDCVEKKDSPEVYFCCCEGNMCNEKFSYFPEMEVTQPTS

SEQ ID NO: 81 - protein, 109 aa, Artificial Sequence
  Synthetic Construct
GAILGRSETQECLFFNANWEKDRTNQTGVEPCYGDKDKARHCFATWKNISGSIEIVKQGCWLDDINCYDRTDCVEKKDSPEVYFCCCEGNMCNEKFSYFPEMEVTQPTS

SEQ ID NO: 82 - protein, 109 aa, Artificial Sequence
  Synthetic Construct
GAILGRSETQECLFFNANWEKDRTNQTGVEPCYGDKDKRRHCFATWKNISGSIEIVAQGCWLDDINCYDRTDCVEKKDSPEVYFCCCEGNMCNEKFSYFPEMEVTQPTS

SEQ ID NO: 83 - protein, 109 aa, Artificial Sequence
  Synthetic Construct
GAILGRSETQECLFFNANWEKDRTNQTGVEPCYGDKDKRRHCFATWKNISGSIEIVYQGCWLDDINCYDRTDCVEKKDSPEVYFCCCEGNMCNEKFSYFPEMEVTQPTS

SEQ ID NO: 84 - protein, 109 aa, Artificial Sequence
  Synthetic Construct
GAILGRSETQECLFFNANWEKDRTNQTGVEPCYGDKDKRRHCFATWKNISGSIEIVFQGCWLDDINCYDRTDCVEKKDSPEVYFCCCEGNMCNEKFSYFPEMEVTQPTS

SEQ ID NO: 85 - protein, 109 aa, Artificial Sequence
  Synthetic Construct
GAILGRSETQECLFFNANWEKDRTNQTGVEPCYGDKDKRRHCFATWKNISGSIEIVIQGCWLDDINCYDRTDCVEKKDSPEVYFCCCEGNMCNEKFSYFPEMEVTQPTS

SEQ ID NO: 86 - protein, 109 aa, Artificial Sequence
  Synthetic Construct
GAILGRSETQECLFFNANWEKDRTNQTGVEPCYGDKDKRRHCFATWKNISGSIEIVKQGCALDDINCYDRTDCVEKKDSPEVYFCCCEGNMCNEKFSYFPEMEVTQPTS

SEQ ID NO: 87 - protein, 109 aa, Artificial Sequence
  Synthetic Construct
GAILGRSETQECLFFNANWEKDRTNQTGVEPCYGDKDKRRHCFATWKNISGSIEIVKQGCWADDINCYDRTDCVEKKDSPEVYFCCCEGNMCNEKFSYFPEMEVTQPTS

SEQ ID NO: 88 - protein, 109 aa, Artificial Sequence
  Synthetic Construct
GAILGRSETQECLFFNANWEKDRTNQTGVEPCYGDKDKRRHCFATWKNISGSIEIVKQGCWLKDINCYDRTDCVEKKDSPEVYFCCCEGNMCNEKFSYFPEMEVTQPTS

SEQ ID NO: 89 - protein, 109 aa, Artificial Sequence
  Synthetic Construct
GAILGRSETQECLFFNANWEKDRTNQTGVEPCYGDKDKRRHCFATWKNISGSIEIVKQGCWLRDINCYDRTDCVEKKDSPEVYFCCCEGNMCNEKFSYFPEMEVTQPTS

SEQ ID NO: 90 - protein, 109 aa, Artificial Sequence
  Synthetic Construct
GAILGRSETQECLFFNANWEKDRTNQTGVEPCYGDKDKRRHCFATWKNISGSIEIVKQGCWLADINCYDRTDCVEKKDSPEVYFCCCEGNMCNEKFSYFPEMEVTQPTS

SEQ ID NO: 91 - protein, 109 aa, Artificial Sequence
  Synthetic Construct
GAILGRSETQECLFFNANWEKDRTNQTGVEPCYGDKDKRRHCFATWKNISGSIEIVKQGCWLFDINCYDRTDCVEKKDSPEVYFCCCEGNMCNEKFSYFPEMEVTQPTS

SEQ ID NO: 92 - protein, 109 aa, Artificial Sequence
  Synthetic Construct
GAILGRSETQECLFFNANWEKDRTNQTGVEPCYGDKDKRRHCFATWKNISGSIEIVKQGCWLGDINCYDRTDCVEKKDSPEVYFCCCEGNMCNEKFSYFPEMEVTQPTS

SEQ ID NO: 93 - protein, 109 aa, Artificial Sequence
  Synthetic Construct
GAILGRSETQECLFFNANWEKDRTNQTGVEPCYGDKDKRRHCFATWKNISGSIEIVKQGCWLMDINCYDRTDCVEKKDSPEVYFCCCEGNMCNEKFSYFPEMEVTQPTS

SEQ ID NO: 94 - protein, 109 aa, Artificial Sequence
  Synthetic Construct
GAILGRSETQECLFFNANWEKDRTNQTGVEPCYGDKDKRRHCFATWKNISGSIEIVKQGCWLNDINCYDRTDCVEKKDSPEVYFCCCEGNMCNEKFSYFPEMEVTQPTS

SEQ ID NO: 95 - protein, 109 aa, Artificial Sequence
  Synthetic Construct
GAILGRSETQECLFFNANWEKDRTNQTGVEPCYGDKDKRRHCFATWKNISGSIEIVKQGCWLIDINCYDRTDCVEKKDSPEVYFCCCEGNMCNEKFSYFPEMEVTQPTS

SEQ ID NO: 96 - protein, 109 aa, Artificial Sequence
  Synthetic Construct
GAILGRSETQECLFFNANWEKDRTNQTGVEPCYGDKDKRRHCFATWKNISGSIEIVKQGCWLDDANCYDRTDCVEKKDSPEVYFCCCEGNMCNEKFSYFPEMEVTQPTS

SEQ ID NO: 97 - protein, 225 aa, Homo sapiens
THTCPPCPAPELLGGPSVFLFPPKPKDTLMISRTPEVTCVVVDVSHEDPEVKFNWYVDGVEVHNAKTKPREEQYNSTYRVVSVLTVLHQDWLNGKEYKCKVSNKALPVPIEKTISKAKGQPREPQVYTLPPSREEMTKNQVSLTCLVKGFYPSDIAVEWESNGQPENNYKTTPPVLDSDGPFFLYSKLTVDKSRWQQGNVFSCSVMHEALHNHYTQKSLSLSPGK

SEQ ID NO: 98 - protein, 4 aa, Artificial Sequence
  Synthetic Construct
GGGA

SEQ ID NO: 99 - protein, 4 aa, Artificial Sequence
  Synthetic Construct
GGGS

SEQ ID NO: 100 - protein, 4 aa, Artificial Sequence
  Synthetic Construct
GGGG

SEQ ID NO: 101 - protein, 5 aa, Artificial Sequence
  Synthetic Construct
GGGGA

SEQ ID NO: 102 - protein, 5 aa, Artificial Sequence
  Synthetic Construct
GGGGS

SEQ ID NO: 103 - protein, 5 aa, Artificial Sequence
  Synthetic Construct
GGGGG

SEQ ID NO: 104 - protein, 4 aa, Artificial Sequence
  Synthetic Construct
GGAG

SEQ ID NO: 105 - protein, 4 aa, Artificial Sequence
  Synthetic Construct
GGSG

SEQ ID NO: 106 - protein, 4 aa, Artificial Sequence
  Synthetic Construct
AGGG

SEQ ID NO: 107 - protein, 4 aa, Artificial Sequence
  Synthetic Construct
SGGG

SEQ ID NO: 108 - protein, 4 aa, Artificial Sequence
  Synthetic Construct
GAGA

SEQ ID NO: 109 - protein, 4 aa, Artificial Sequence
  Synthetic Construct
GSGS

SEQ ID NO: 110 - protein, 6 aa, Artificial Sequence
  Synthetic Construct
GAGAGA

SEQ ID NO: 111 - protein, 6 aa, Artificial Sequence
  Synthetic Construct
GSGSGS

SEQ ID NO: 112 - protein, 8 aa, Artificial Sequence
  Synthetic Construct
GAGAGAGA

SEQ ID NO: 113 - protein, 8 aa, Artificial Sequence
  Synthetic Construct
GSGSGSGS

SEQ ID NO: 114 - protein, 10 aa, Artificial Sequence
  Synthetic Construct
GAGAGAGAGA

SEQ ID NO: 115 - protein, 10 aa, Artificial Sequence
  Synthetic Construct
GSGSGSGSGS

SEQ ID NO: 116 - protein, 12 aa, Artificial Sequence
  Synthetic Construct
GAGAGAGAGAGA

SEQ ID NO: 117 - protein, 12 aa, Artificial Sequence
  Synthetic Construct
GSGSGSGSGSGS

SEQ ID NO: 118 - protein, 6 aa, Artificial Sequence
  Synthetic Construct
GGAGGA

SEQ ID NO: 119 - protein, 6 aa, Artificial Sequence
  Synthetic Construct
GGSGGS

SEQ ID NO: 120 - protein, 9 aa, Artificial Sequence
  Synthetic Construct
GGAGGAGGA

SEQ ID NO: 121 - protein, 9 aa, Artificial Sequence
  Synthetic Construct
GGSGGSGGS

SEQ ID NO: 122 - protein, 12 aa, Artificial Sequence
  Synthetic Construct
GGAGGAGGAGGA

SEQ ID NO: 123 - protein, 12 aa, Artificial Sequence
  Synthetic Construct
GGSGGSGGSGGS

SEQ ID NO: 124 - protein, 8 aa, Artificial Sequence
  Synthetic Construct
GGAGGGAG

SEQ ID NO: 125 - protein, 8 aa, Artificial Sequence
  Synthetic Construct
GGSGGGSG

SEQ ID NO: 126 - protein, 12 aa, Artificial Sequence
  Synthetic Construct
GGAGGGAGGGAG

SEQ ID NO: 127 - protein, 12 aa, Artificial Sequence
  Synthetic Construct
GGSGGGSGGGSG

SEQ ID NO: 128 - protein, 15 aa, Artificial Sequence
  Synthetic Construct
GGGGAGGGGAGGGGA

SEQ ID NO: 129 - protein, 15 aa, Artificial Sequence
  Synthetic Construct
GGGGSGGGGSGGGGS

SEQ ID NO: 130 - protein, 5 aa, Artificial Sequence
  Synthetic Construct
GGGAG

SEQ ID NO: 131 - protein, 6 aa, Artificial Sequence
  Synthetic Construct
GGGAGG

SEQ ID NO: 132 - protein, 7 aa, Artificial Sequence
  Synthetic Construct
GGGAGGG

SEQ ID NO: 133 - protein, 4 aa, Artificial Sequence
  Synthetic Construct
AAAL

SEQ ID NO: 134 - protein, 4 aa, Artificial Sequence
  Synthetic Construct
AAAK

SEQ ID NO: 135 - protein, 4 aa, Artificial Sequence
  Synthetic Construct
AAAR

SEQ ID NO: 136 - protein, 14 aa, Artificial Sequence
  Synthetic Construct
EGKSSGSGSESKST

SEQ ID NO: 137 - protein, 12 aa, Artificial Sequence
  Synthetic Construct
GSAGSAAGSGEF

SEQ ID NO: 138 - protein, 12 aa, Artificial Sequence
  Synthetic Construct
AEAAAKEAAAKA

SEQ ID NO: 139 - protein, 18 aa, Artificial Sequence
  Synthetic Construct
KESGSVSSEQLAQFRSLD

SEQ ID NO: 140 - protein, 10 aa, Artificial Sequence
  Synthetic Construct
GENLYFQSGG

SEQ ID NO: 141 - protein, 8 aa, Artificial Sequence
  Synthetic Construct
SACYCELS

SEQ ID NO: 142 - protein, 5 aa, Artificial Sequence
  Synthetic Construct
RSIAT

SEQ ID NO: 143 - protein, 17 aa, Artificial Sequence
  Synthetic Construct
RPACKIPNDLKQKVMNH

SEQ ID NO: 144 - protein, 36 aa, Artificial Sequence
  Synthetic Construct
GGSAGGSGSGSSGGSSGASGTGTAGGTGSGSGTGSG

SEQ ID NO: 145 - protein, 17 aa, Artificial Sequence
  Synthetic Construct
AAANSSIDLISVPVDSR

SEQ ID NO: 146 - protein, 36 aa, Artificial Sequence
  Synthetic Construct
GGSGGGSEGGGSEGGGSEGGGSEGGGSEGGGSGGGS

SEQ ID NO: 147 - protein, 5 aa, Artificial Sequence
  Synthetic Construct
EAAAK

SEQ ID NO: 148 - protein, 5 aa, Artificial Sequence
  Synthetic Construct
PAPAP

SEQ ID NO: 149 - protein, 115 aa, Artificial Sequence
  Synthetic Construct
GRGEAETRECIFYNANWEKDRTNQSGLEPCYGDQDKRRHCFASWKNSSGTIELVKQGCWLDDINCYDRQECVAKKDSPEVYFCCCEGNFCNERFTHLPEAGGPEVTYEPPPTAPT

SEQ ID NO: 150 - protein, 109 aa, Artificial Sequence
  Synthetic Construct
GAILGRSETQECLFYNANWELERTNQTGVERCEGEKDKRLHCYATWRNISGSIEIVAKGCWLDDFNCYDRTDCVETEENPQVYFCCCEGNMCNEKFSYFPEMEVTQPTS

SEQ ID NO: 151 - protein, 246 aa, Homo sapiens
MEWSWVFLFFLSVTTGVHSDKTHTCPPCPAPELLGGPSVFLFPPKPKDTLMISRTPEVTCVVVDVSHEDPEVKFNWYVDGVEVHNAKTKPREEQYNSTYRVVSVLTVLHQDWLNGKEYKCKVSNKALPAPIEKTISKAKGQPREPQVYTLPPSRDELTKNQVSLTCLVKGFYPSDIAVEWESNGQPENNYKTTPPVLDSDGSFFLYSKLTVDKSRWQQGNVFSCSVMHEALHNHYTQKSLSLSPGK

SEQ ID NO: 152 - protein, 11 aa, Artificial Sequence
  Synthetic Construct
DICLPRWGCLW

SEQ ID NO: 153 - protein, 93 aa, Homo sapiens
GPVEVFITETPSQPNSHPIQWNAPQPSHISKYILRWRPKNSVGRWKEATIPGHLNSYTIKGLKPGVVYEGQLISIQQYGHQEVTRFDFTTTST

SEQ ID NO: 154 - protein, 609 aa, Homo sapiens [sequence omitted]

SEQ ID NO: 155 - protein, 6 aa, Homo sapiens
NPVTPK